European Patent Specification EP 4 204 393 B1, published July 29, 2026. Title: Aminocarbamoyl compounds for the treatment of viral infections. Applicant: F. Hoffmann-La Roche AG. The sequence listing filed with the application follows.

SEQUENCE LISTING (6 sequences)

SEQ ID NO: 1 - protein, 306 aa, SARS-CoV-2 [sequence omitted]

SEQ ID NO: 2 - protein, 306 aa, SARS-CoV
SGFRKMAFPSGKVEGCMVQVTCGTTTLNGLWLDDTVYCPRHVICTAEDMLNPNYEDLLIRKSNHSFLVQAGNVQLRVIGHSMQNCLLRLKVDTSNPKTPKYKFVRIQPGQTFSVLACYNGSPSGVYQCAMRPNHTIKGSFLNGSCGSVGFNIDYDCVSFCYMHHMELPTGVHAGTDLEGKFYGPFVDRQTAQAAGTDTTITLNVLAWLYAAVINGDRWFLNRFTTTLNDFNLVAMKYNYEPLTQDHVDILGPLSAQTGIAVLDMCAALKELLQNGMNGRTILGSTILEDEFTPFDVVRQCSGVTFQ

SEQ ID NO: 3 - protein, 15 aa, Artificial Sequence
  Synthetic Construct
KTSAVLQSGFRKMEK

SEQ ID NO: 4 - protein, 306 aa, MERS-CoV
SGLVKMSHPSGDVEACMVQVTCGSMTLNGLWLDNTVWCPRHVMCPADQLSDPNYDALLISMTNHSFSVQKHIGAPANLRVVGHAMQGTLLKLTVDVANPSTPAYTFTTVKPGAAFSVLACYNGRPTGTFTVVMRPNYTIKGSFLCGSCGSVGYTKEGSVINFCYMHQMELANGTHTGSAFDGTMYGAFMDKQVHQVQLTDKYCSVNVVAWLYAAILNGCAWFVKPNRTSVVSFNEWALANQFTEFVGTQSVDMLAVKTGVAIEQLLYAIQQLYTGFQGKQILGSTMLEDEFTPEDVNMQIMGVVMQ

SEQ ID NO: 5 - protein, 302 aa, HCoV-229E
AGLRKMAQPSGFVEKCVVRVCYGNTVLNGLWLGDIVYCPRHVIASNTTSAIDYDHEYSIMRLHNFSIISGTAFLGVVGATMHGVTLKIKVSQTNMHTPRHSFRTLKSGEGFNILACYDGCAQGVFGVNMRTNWTIRGSFINGACGSPGYNLKNGEVEFVYMHQIELGSGSHVGSSFDGVMYGGFEDQPNLQVESANQMLTVNVVAFLYAAILNGCTWWLKGEKLFVEHYNEWAQANGFTAMNGEDAFSILAAKTGVCVERLLHAIQVLNNGFGGKQILGYSSLNDEFSINEVVKQMFGVNLQ

SEQ ID NO: 6 - protein, 302 aa, HCoV-OC43
SGIVKMVNPTSKVEPCVVSVTYHNMTLNGLWLDDKVYCPRHVICSASDMTNPDYTNLLCVTSSDFTVLFDRLSLTVMSYQMRGCMLVLTVTLQNSRTPKYTFGVVKPGETFTVLAAYNGKPQGAFHVTMRSSYTIKGSFLCGSCGSVGYVIMGDCVKFVYMHQLELSTGCHTGTDFNGDFYGPYKDAQVVQLPIQDYIQSVNFLAWLYAAILNNCNWFIQSDKCSVEDFNVMALSNGFSQVKSDLVIDALASMTGVSLETLLAAIKRLKNGFQGRQIMGSCSFEDELTPSDVYQQLAGIKLQ